European Patent Specification EP 3 512 557 B1, published September 25, 2024. Title: Combinations including ABX196 for the treatment of cancer. Applicant: ABIVAX. The sequence listing filed with the application follows.

SEQUENCE LISTING (4 sequences)

SEQ ID NO: 1 - protein, 31 aa, Artificial Sequence
  Amino acid sequence of peptide Cl II- TRP2(180-188)
KFGWTGPDCNRKKPAGGNCSVYDFFVWLHYY

SEQ ID NO: 2 - protein, 15 aa, Artificial Sequence
  Amino acid sequence of Class II epitope
KFGWTGPDCNRKKPA

SEQ ID NO: 3 - protein, 9 aa, Artificial Sequence
  Amino acid sequence of an immunodominant peptide from the tumor associated antigen tyrosinase-related protein-2
SVYDFFVWL

SEQ ID NO: 4 - protein, 32 aa, Artificial Sequence
  Amino acid sequence of a peptide comprising the sequence of an immunodominant peptide from TRP2
GGGSVYDFFVWLGGGSSKFGWTGPDCNRKKPA